European Patent Specification EP 3 237 908 B1, published April 22, 2026. Title: Directed evolution of membrane proteins in eukaryotic cells with a cell wall. Applicant: Universität Zürich. The sequence listing filed with the application follows.

SEQUENCE LISTING (33 sequences)

SEQ ID NO: 1 - DNA, 50 bp, Artificial Sequence
  Fwd primer for error prone PCR
ctaaagaagaaggggtatctctcgagaaacgtgaggcggaagcggctagc

SEQ ID NO: 2 - DNA, 50 bp, Artificial Sequence
  Reverse primer for error prone PCR
attacatgactcgactcgatgccgacgagagcggccgcctattaggatcc

SEQ ID NO: 3 - protein, 6 aa, Artificial Sequence
  labelled Neurotensin
  MISC_FEATURE (1)..(1): labelled with HiLyte Fluor 488
KKPYIL

SEQ ID NO: 4 - protein, 11 aa, Artificial Sequence
  Substance P from Homo sapiens modified
  MISC_FEATURE (3)..(3): labeled with HiLyte Fluor 488
RPKPQQFFGLM

SEQ ID NO: 5 - protein, 11 aa, Artificial Sequence
  Dynorphin A from homo sapiens modified
  MISC_FEATURE (11)..(11): labeled with HiLyte Fluor 488
YGGFLRRIRPK

SEQ ID NO: 6 - protein, 424 aa, Rattus norvegicus
MHLNSSVPQGTPGEPDAQPFSGPQSEMEATFLALSLSNGSGNTSESDTAGPNSDLDVNTDIYSKVLVTAIYLALFVVGTVGNSVTAFTLARKKSLQSLQSTVHYHLGSLALSDLLILLLAMPVELYNFIWVHHPWAFGDAGCRGYYFLRDACTYATALNVASLSVERYLAICHPFKAKTLMSRSRTKKFISAIWLASALLAIPMLFTMGLQNRSGDGTHPGGLVCTPIVDTATVKVVIQVNTFMSFLFPMLVISILNTVIANKLTVMVHQAAEQGRVCTVGTHNGLEHSTFNMTIEPGRVQALRHGVLVLRAVVIAFVVCWLPYHVRRLMFCYISDEQWTTFLFDFYHYFYMLTNALFYVSSAINPILYNLVSANFRQVFLSTLACLCPGWRHRRKKRPTFSRKPNSMSSNHAFSTSATRETLY

SEQ ID NO: 7 - protein, 424 aa, Rattus norvegicus
MHLNSSVPQGTPGEPDAQPFSGPQSEMEATFLALSLSNGSGNTSESDTPGPNSDLDVNTDIYSKVLVTAIYLALFVVGTVGNSVTAFTLARKKSLQSLQSTVHYHLGSLALSNLLILLLAMPVELYNFIWVHHPWAFGDAGCRGYYFLRDACTYATALNVASLSVERYLAICHPFKAKTLMSRSRTKKFISAIWLASALLAIPMLFTMGLQNRSGDGTHPGGLVCTPIVDTATVKVVIQVNTFMSFLFPMLVISILNTVISNKLTVMVHQAAEQGRVCTVGTHNGLEHSTFNMTIEPGRVQALRHGVLVLRAVVIAFVVCWLPYHVRRLMFCYISDEQWTTFLFDFYHYFYMLTNSLFYVSSAINPILYNLVSANFRQVFLSTLACLCPGWRHRRKKRPTFSRKPNSMSSNHAFSTSATRETLY

SEQ ID NO: 8 - protein, 424 aa, Rattus norvegicus
MHLNSSVPQGTPGEPDAQPFSGPQSEMEATFLALSLSNGSGNTSESDTPGPNSDLDVNTDIYSKVLVTAIYLALFVVGTVGNSVTAFTLARKKSLQSLQSTVHYHLGSLALSNLLILLLAMPVELYNFIWVHHPWAFGDAGCRGYYFLRDACTYATALNVASLSVERYLAICHPFKAKTLMSRSRTKKFISAIWLASALLAIPMLFTMGLQNRSGDGTHPGGLVCTPIVDTATVKVVIQVNTFMSFLLPMLVISILNTVISNKLTVMVHQAAEQGRVCTAGTHNGLEHSTFNMTIEPGRVQALRHGVLVLRAVVIAFVVCWLPYHVRRLMFCYISDEQWTTFLFDFYHYFYMLTNSLFYVSSAINPILYNLVSANFRQVFLSTLACLCPGWRHRRKKRPTFSRKPNSMSSNHAFSTSATRETLY

SEQ ID NO: 9 - protein, 424 aa, Rattus norvegicus; identical to SEQ ID NO: 6

SEQ ID NO: 10 - protein, 424 aa, Rattus norvegicus
MHLNSSVPQGTPGEPDAQPFSGPQSEMEATFLALSLSNGSGNTSESDTPGPNSDLDVNTDIYSKVLVTAIYLALFVVGTVGNSVTAFTLARKKSLQSLQSTVHYHLGSLALSNLLILLLAMPVELYNFIWVHHPWAFGDAGCRGYYFLRDACTYATALNVASLSVERYLAICHPFKAKTLMSRSRTKKFISAIWLASALLAIPMLFTMGLQNRSGDGTHPGGLVCTPIVDTATVKVVIQVNTFMSFLFPMLVISILNTVISNKLTVMVHQAAEQGRVCTVGTHNGLEHSTFNMTIEPGRVQALRHGVLVLRAVVIAFVVCWLPYHVRRLMFCYISDEQWTTFLFDFYHYFYMLTNSLFYVSSAINPILYNLVSANFRQVFLSTLACLCPGWRHRRKKWPTFSRKPNSMSSNHAFSTSATRETLY

SEQ ID NO: 11 - protein, 424 aa, Rattus norvegicus
MHLNSSVPQGTPGEPDAQPFSGPQSEMEATFLALSLSNGSGNTSESDTPGPNSDLDVNTDIYSKVLVTAIYLALFVVGTVGNSVTAFTLARKKSLQSLQSTVHYHLGSLALSNLLILLLAMPVELYNFIWVHHPWAFGDAGCRGYYFLRDACTYATALNVASLSVERYLAICHPFKAKTLMSRSRTKKFISAIWLASALLAIPMLFTMGLQNRSGDGTHPGGLVCTPIVDTATVKVVIQVNTFMSFLFPMLVISILNTVISNKLTVMVHQAAEQGRVCTVGTHNGLEHSTFNMTIEPGRVQALRHGVLVLRAVVIAFVVCWLPYHVRRLMFCYISDEQWTTFLFDFYHYFYMLTNSLFYVSSAINPILYNLVSANFRQVFLSTLAGLCPGWCHRRKKRPTFSRKPNSMSSNHAFSTSATRETLY

SEQ ID NO: 12 - protein, 424 aa, Rattus norvegicus
MHLNSSVPQGTPGEPDAQPFSGPQSEMEATFLALSLSNGSGNTSESDTPGPNSDLDVNTDIYSKVLVTAIYLALFVVGTVGNSVTAFTLARKKSLQSLQSTVHYHLGSLALSNLLILLLAMPVELYNFIWVHHPWAFGDAGCRGYYFLRDACTYATALNVASLSVERYLAICHPFKAKTLMSRSRTKKFISAIWLASALLAIPMLFTMGLQNRSGDGTHPGGLVCTPIVDTATVKVVIQVNTFMSFLFPMLVISILSTVISNKLTVMVHQAAEQGRVCTVGTHDGLEHSTFNMTIEPGRVQALRHGVLVLRAVVIAFVVCWLPYHVRRLMFCYISDEQWTTFLFDFYHYFYMLTNTLLYVSSTINPILYILVSANFRQVFLSTLACLCPGWCHRRKKRPTFSRKPNSMSSNHAFSTSATRETLY

SEQ ID NO: 13 - protein, 424 aa, Rattus norvegicus
MHLNSSVPQGTPGEPDAQPFSGPQSEMEATFLALSLSNGSGNTSESDTPGPNSDLDVNTDIYSKVLVTAIYLALFVVGTVGNSVTAFTLARKKSLQSLQSTVHYHLGSLALSNLLILLLAMPVELYNFIWVHHPWAFGDAGCRGYYFLRDACTYATALNVASLSVERYLAICHPFKAKTLMSRSRTKKFISALWLASALLAIPMLFTMGLQNRSGDGTHPGGLVCTPIVDTATVKVAIQVNTFMSFLFPMLVISILNTVISNKLTVMGHQAAEQGRVCTVGTHNGLEHSTFDMTIEPGRVQALRHGVLVLRAVVIAFAVCWLPYHVRRLMFCYISDEQWTTFLFDFYHYFYMLTNTLLYVSSAINPILYILVSANFRQAFLSTLACLCPGWCHRRKKRPTFSRKPNSMSSNHAFSTSATRETLY

SEQ ID NO: 14 - protein, 407 aa, Homo sapiens
MDNVLPVDSDLSPNISTNTSEPNQFVQPAWQIVLWAAAYTVIVVTSVVGNVVVMWIILAHKRMRTVTNYFLVNLAFAEASMAAFNTVVNFTYAVHNEWYYGLFYCKFHNFFPIAAVFASIYSMTAVAFDRYMAIIHPLQPRLSATATKVVICVIWVLALLLAFPQGYYSTTETMPSRVVCMIEWPEHPNKIYEKVYHICVTVLIYFLPLLVIGYAYTVVGITLWASEIPGDSSDRYHEQVSAKRKVVKMMIVVVCTFAICWLPFHIFFLLPYINPDLYLKKFIQQVYLAIMWLAMSSTMYNPIIYCCLNDRFRLGFKHAFRCCPFISAGDYEGLEMKSTRYLQTQGSVYKVSRLETTISTVVGAHEEEPEDGPKATPSSLDLTSNCSSRSDSKTMTESFSFSSNVLS

SEQ ID NO: 15 - protein, 407 aa, Homo sapiens
MDNVLPVDSDLSPNISTNTSEPNQFVQPAWQIVLWAAAYTVIVVTSVVGNVVVMWIILAHKRMRTVTNYFLVNLAFAEASMAAFNTVVNFTYAVHNEWYYGLFYCKFHNFFPIAAVFASIYSMTAVAFDRYMAIIHPLQPRLSATATKVVICVIWVLALLLAFPQGYYSTTETMPSRVVCMIEWPEHPNKIYEKVYHICVTVLIYFLPLLVIGYAYTVVGITLWASEIPGDSSDRYHEQVSAKRKVVKMMIVVVCTFAICWLPFHIFFLLPYINPDLYLKKFIQQVYLAIMWLAMSSTMYNPIIYCCLNDRFRLGFKHAFRCCPFISAGDYEGLKMKSTRYLQTQGSVYKVSRLETTISTVVGAHEEEPEDGPKATPSSLDLTSNCSSRSDSKTMTESFSFSSNVLS

SEQ ID NO: 16 - protein, 407 aa, Homo sapiens
MDNVLPVDSDLSPNISTNTSEPNQFVQPAWQIVLWAAAYTVIVVTSVVGNVVVMWIILAHKRMRTVTNYFLVNLAFAEASMAAFNTVVNFTYAVHNEWYYGLFYCKFHNFFPIAAVFASIYSMTAVAFDRYMAIIHPLQPRLSATATKVVICVIWVLALLLAFPQGYYSTTETMPSRVVCMIEWPEHPNKIYEKVYHICVTVLIYFLPLLVIGYAYSVVGITLWASEIPGDSSDRYHEQVSAKRKVVKMMIVVVCTFAICWLPFHIFFLLPYINPDLYLKKFIQQAYLAIMWLAMSSTMYNPIIYCCLNDRFRLGFKHAFRCCPFISAGDYEGLEMKSTRYLQTQGSVYKVSRLETTISTVVGAHEEEPEDGPKATPSSLDLTSNCSSRSDSKTMTESFSFSSNVLS

SEQ ID NO: 17 - protein, 407 aa, Homo sapiens
MDNVLPVDSDLSPNISTNTSEPNQFVQPAWQIVLWAAAYTVIVVTSVVGNVVVMWIILAHKRMRTVTNYFLVNLAFAEASMAAFNTVVNFTYAVHNEWYYGLFYCKFHNFFPIAAVFASIYSMTAVAFDRYMAIIHPLQPRLSATATKVVICVIWVLALLLAFPQGYYSTTETMPSRVVCMIEWPEHPNKIYEKVYHICVTVLIYFLPLLVIGYAYTVVGITLWASEIPGDSSDRYHEQVSAKRKVVKMMIVVVCTFAICWLPFHIFFLLPYIYPDLYLKKFIQQVYLAIMWLAMSSTMYNPIIYCCLNDRFRLGFKHAFRCCPFISAGDYEGLEMKSTRYLQTQGSVYKVSRLETTISTVVGAHEEEPEDGPKATPSSLDLTSNCSSRSDSKTMTESFSFSSNVLS

SEQ ID NO: 18 - protein, 407 aa, Homo sapiens; identical to SEQ ID NO: 14

SEQ ID NO: 19 - protein, 407 aa, Homo sapiens
MDNVLPVDSDLSPNISTNTSEPNQFVQPAWQIVLWAAAYTVIVVTSVVGNVVVMWIILAHKRMRTVTNYFLVNLAFAEASMAAFNTVVNFTYAVHNEWYYGLFYCKFHNFFPIAAIFASIYSMTAVAFDRYMAIIHPLQPRLSATATKVVICVIWVLALLLAFPQGYYSTTETMPSRVVCKIEWPEHPNKIYEKVYHICVTVLIYFLPLLVIGYAYTVVGITLRASEIPGDSSDRYHEQVSAKRKVVKMMIVVVCTFAICWLPFHIFFLLPYINPDLYLKKFIQQVYLAIMWLAMSSTMYNPIIYCCLNDRFRLGFKHAFRCCPFISAGDYEGLEMKSTRYLQTQGSVYKVSRLETTISTVVGAHEEEPEDGPKATPSSLDLTSNCSSRSDSKTMTESFSFSSNVLS

SEQ ID NO: 20 - protein, 407 aa, Homo sapiens
MDNVLPVDSDLSPNISTNTSEPNQFVQPAWQIVLWAAAYTVIVVTSVVGNVVVMWIILAHKRMRTVTNYFLVNLAFAEASMAAFNTVVNFTYAVHNEWYYGLFYCKFHNFFPIAAIFASIYSMTAVAFDRYMAIIHPLQPRLSATATKVVICVIWVLALLLAFPQGYYSTTETMPSRVVCKIEWPEHPNKIYEKVYHICVTVLIYFLPLLVIGYAYTVVGITLRASEIPGDSSDRYHEQVSAKRKVVKMMIVVVCTFAICWLPFHIFFLLPYINPDLYLKKFIQQVYLAIMWLAMSSTMYNPIIYCCLNDRFRLGFKHAFRWCPFISAGDYEGLKMKSTRYLQTQGSVYKVSRLETTISTVVGAHEEEPEDGPKATPSSLDLTSNCSSRSDSKTMTESFSFSSNVLS

SEQ ID NO: 21 - protein, 407 aa, Homo sapiens
MDNVLPVDSDLSPNISTNTSEPNQFVQPAWQIVLWAAAYAVIVVTSVVGNVVVMWIILAHKRMRTVTNYFLVNLAFAEASMAAFNTVVNFTYAVHNEWYYGLFYCKFHNFFPIAAIFASIYSMTAVAFDRYMAIIHPLQPRLSATATKVVICVIWVLALLLAFPQGYYSTTETMPSRVVCKIEWPEHPNKIYEKVYHICVTVLIYFLPLLVIGYAYTVVGITLRASEIPGDSSDRYHEQVSAKRKVVKMMIVVVCTFAICWLPFHIFFLLPYINPDLYLKKFIQQVYLAIMWLAMSSTMYNPIIYCCLNDRFRLGFKHAFRWCPFISAGDYEGLKMKSTRYLQTQGSVYKVSRLETTISTVVGAHEEEPEDGPKATPSSLDLTSNCSSRSDSKTMTESFSFSSNVLS

SEQ ID NO: 22 - protein, 407 aa, Homo sapiens
MDNVLPVDSDLSPNISTNTSEPNQFVQPAWQIVLWAAAYTVIVVTSVVGNVVVMWIILAHKRMRTVTNYFLVNLAFAEASMAAFNTVVNFTYAVHNEWYYGLFYCKFHNFFPIAAIFASIYSMTAVAFDRYMAIIHPLQPRLSATATKVVICVIWVLALLLAFPQGYYSTTETMPSRVVCKIEWPEHPNKIYEKVYHICVTVLIYFLPLLVIGYAYTVVGITLWASEIPGDSSDRYHEQVSAKRKVVKMMIVVVCTFAICWLPFHIFFLLPYINPDLYLKKFIQQVYLAIMWLAMSSTMYNPIIYCCLNDRFRLGFKHAFRWCPFISAGDYEGLKMKSTRYLQTQGSVYKVSRLETTISTVVGAHEEEPEDGPKATPSSLDLTSNCSSRSDSKTMTESFSFSSNVLS

SEQ ID NO: 23 - protein, 407 aa, Homo sapiens
MDNVLPVDSDLSPNISTNTSEPNQFVQPAWQIVLWAAAYAVIVVTSVVGNVVVMWIILAHKSMRTVTNYFLVNLAFAEASMAAFNTVVNFTYAVHNEWYYGLFYCKFHNFFPIAAVFASIYSMTAVAFDRYMAIIHPLQPRLSATATKVVICVIWVLALLLAFPQGYYSTTETMPSRVVCMIEWPEHPNKIYEKVYHICVTVLIYFLPLLVIGYAYTVVGITLWASEIPGDSSDRYHEQVSAKRKVVKMMIVVVCTFAICWLPYHIFFLLPYINPDLYLKKFIQQVYLAIMWLAMSSTTYNPIIYCCLNDRFRLGFKHAFRCCPFISAGDYEGLEMKSTRYLQTQGSVYKVSRLETTISTVVGAHEEEPEDGPKATPSSLDLTSNCSSRSDSKTMTESFSFSSNVLS

SEQ ID NO: 24 - protein, 407 aa, Homo sapiens
MDNVLPVDSDLSPNISTNTSEPNQFVQPAWQIVLWAAAYTVIVVTSVVGNVVVMWIILAHKRMRTVTNYFLVNLAFAEASMAAFNTVVNFTYAVRNEWYYGLFYCKFHNFFPIAAVFASIYSMTAVAFDRYMAIIHPHQPRLSATATKVVICVIWVLALLLAFPQGYYSTTETMPSRVVCKIEWPEHPNKIYEKVYHICVTVLIYFLPLLVIGYAYTVVGITLRASEIPGDSSDRYHEQVSAKRKVVKMMIVVVCTFAICWLPFHIFFLLPYINPDLFLKKFIQQVYLAIMWLAMSSTMYNPIIYCCLNDRFRLGFKHAFRWCPFISAGDYEGLKMKSTRYLQTQGSVYKVSRLETTISTVVGAHEEEPEDGPKATPSSLDLTSNCSSRSDSKTMTESFSFSSNVLS

SEQ ID NO: 25 - protein, 407 aa, Homo sapiens
MDNVLPVDSDLSPNISTNTSEPNQFVQPAWQIVLWAAAYTVIVVTSVVGNVVVMWIILAHKRMRTVTNYFLVNLAFAEASMAAFNTVVNFTYAVHNEWYYGLFYCKFHNFFPIAAVFASIYSMTAVAFVRYMAIIHPLQPRLSATATKVVICVIWVLALLLAFPQGYYSTTETMPSRVVCKIEWPEHPNKIYEKVYHICVTVLIYFLPLLVIGYAYTVVGIRLWASEIPGDSSDRYHEQVSAKRKVVKMMIVVVCTFAICWLPYHIFFLLPYINPDLYLKKFIQQVYLAIMWLAMSSTMYNPIIYCCLNDRFRLGFKHAFRWCPFISAGDYEGLKMKSTRYLQTQGSVYKVSRLETTISTVVGAHEEEPEDGPKATPSSLDLTSNCSSRSDSKTMTESFSFSSNVLS

SEQ ID NO: 26 - protein, 380 aa, Homo sapiens
MDSPIQIFRGEPGPTCAPSACLPPNSSAWFPGWAEPDSNGSAGSEDAQLEPAHISPAIPVIITAVYSVVFVVGLVGNSLVMFVIIRYTKMKTATNIYIFNLALADALVTTTMPFQSTVYLMNSWPFGDVLCKIVISIDYYNMFTSIFTLTMMSVDRYIAVCHPVKALDFRTPLKAKIINICIWLLSSSVGISAIVLGGTKVREDVDVIECSLQFPDDDYSWWDLFMKICVFIFAFVIPVLIIIVCYTLMILRLKSVRLLSGSREKDRNLRRITRLVLVVVAVFVVCWTPIHIFILVEALGSTSHSTAALSSYYFCIALGYTNSSLNPILYAFLDENFKRCFRDFCFPLKMRMERQSTSRVRNTVQDPAYLRDIDGMNKPV

SEQ ID NO: 27 - protein, 380 aa, Homo sapiens
MDSPIQIFRGEPGPTCAPSACLPPNSSAWFPGWAEPDSNGSAGSEDAQLEPAHISPAIPVIITAVYSVVFVVGLVGNSLVMFVIIRYTKMKTATNIYIFNLALADALVTATMPFQSTDYLMNSWPFGDVLCKIVISIDYYSMFTSIFTLTMMCVDRYIAVCHPVKALDFRTPLKAKIINICIWLLSSSVGISAIVLGGTKVREDVDVIECSLQFPDDDYSWWDLFMKICVFIFAFVIPVLIIIVCYTLMILRLKSVRLLSGSREKDRNLRRITRLVLVVVAVFVVCWTPIHIFILVEALGSTSHSTAALSSYYFCIALGYINSSLNPILYAFLDENFKRCFRDFCFPLKMRMKRQSTSRVRNTVQDPAYLRDIDGMNKPV

SEQ ID NO: 28 - protein, 380 aa, Homo sapiens
MDSPIQIFRREPGPTCAPSACLPPNSSAWFPGWAEPDSNGSAGSEDAQLEPAHISPAIPVIITAVYSVVFVVGLVGNSLVMFVIIRYTKMKTATNIYIFSLALAGALVTTTMPFQSTDYLMNSWPFGDVLCKIVISIDYYSMFTSIFTLTMMCVDRYIAVCHPVKALDFRTPLKAKIINICIWLLSSSVGISAIVLGGTKVREDVDVIECSLQFPDDDYSWWDLFMKICVFIFAFVIPVLIIIVCYTLMILRLKSVRLLSGSREKDRNLRRITRLVLVVVAVFVVCWTPIHIFILVEALGGTSHSTAALSSYYFCIALGYINSSLNPILYAFLDENFKRCFRDFCFPLKMRMKRQSTSRVRNTVQDPAYLRDIDGMNKPV

SEQ ID NO: 29 - protein, 380 aa, Homo sapiens
MDSPIQIFRGEPGPTCAPSACLPPNSSAWFPGWAEPDSNGSAGSEDAQLEPAHISPAIPVIITAVYSVVFVVGLVGNSLVMFVIIRYTKMKTATNIYIFSLALAGALVTTTMPFQSTDYLMNSWPFGDVLCKIVISIDYYSMFTSIFTLTMMCVDRYIAVCHPVKALDFRTPLKAKIINICIWLLSSSVGISAIVLGGTKVREDVDVIECSLQFPDDDYSWWDLFMKICVFIFAFVIPVLIIIVCYTLMILRLKSVRLLSGSREKDRNLRRITRLVLVVVAVFVVCWTPIHIFILVEALGSTSHSTAALSSYYFCIALGYINSSLNPILYAFLDENFKRCFRDFCFPLKMRMKRQSTSRVRNTVQDPAYLRDIDGMNKPV

SEQ ID NO: 30 - protein, 380 aa, Homo sapiens
MDSPIQIFRGEPGPTCAPSACLPRNSSAWFPGWAEPDSNGSAGSEDAQLEPAHISPAIPVIITAVYSVVFVVGLVGNSLVMFVIIRYTKMKTATNIYIFSLALAGALVTTTMPFQSTDYLMNSWPFGDVLCKIVISIDYYSMFTSIFTLTMMCVDRYIAVCHPVKALDFRTPLKAKIINICIWLLSSSVGISAIVLGGTKVREDVDVIECSLQFPDDDYSWWDLFMKICVFIFAFVIPVLIIIVCYTLMILRLKSVRLLSGSREKDRNLRRITRLVLVVVAVFVVCWTPIHIFILVEALGSTSHSTAALSSYYFCIALGYINSSLNPILYAFLDENFKRCFRDFCFPLKMRMKRQSTSRVRNTVQDPAYLRDIDGMNKPV

SEQ ID NO: 31 - protein, 380 aa, Homo sapiens
MDSPIQIFRGEPGPTCAPSACLPPNSSAWFPGWAEPDSNGSAGSEDAQLEPAHISPAIPVIITAVYSVVFVVGLVGNSLVMFVIIRYTKMKTATNIYIFSLALAGALVTTTMPFQSTDYLMNSWPFGDVLCKIVISIDYYSMFTSIFTLTMMCVDRYIAVCHPVKALDFRTPLKAKIINICIWLLSSSVGISAIVLGGTKVREDVDVIECSLQFPDDDYSWWDLFMKICVFIFAFVIPVLIIIVCYTLMILRLKSVRLLSGSREKDRNLRRITRLVLVVVVVFVVCWTPIHIFILVEALGSTSHSTAALSSYYFCIALGYINSSLNPILYAFLDENFKRCFRDFCFPLKMRMKRQSTSRVRNTVQDPAYLRDIDGMNKPV

SEQ ID NO: 32 - protein, 380 aa, Homo sapiens
MDSPIQIFRGEPGPTCAPSACLPPNSSAWFPGWAEPDSNGSAGSEDAQLEPAHISPAIPVIITAVYSVVFVVGLVGNSLVMFVIIRYTKMKTATNIYIFSLALAGALVTTTMPFQSTDYLMNSWPFGDVLCKIVISIDYYSMFTSIFTLTMMCVDHYIAVCHPVKALDFRTPLKAKIINICIWLLSSSVGISAIVLGGTKVRDDVDVIECSLQFPDDDYSWWDLFMKICVFIFAFVIPVLIIIVCYTLMILRLKSVRLLSGSREKDRNLRRITRLVLVVVAVFVVCWTPIHIFILVEALGSTSHSTAALSSYYFCIALGYINSSLNPILYAFLDENFKRCFRDFCFPLKMRMKRQSTSRVRNTVQDPAYLRDIDGMNKPV

SEQ ID NO: 33 - protein, 380 aa, Homo sapiens
MDSPIQIIRGEPGPTCAPSACLPPNSSAWFPGWAEPDSNGSAGSEDAQLEPAHIPPAIPVIITAVYSVVFVVGLVGNSLVMFVIIRYTKMKTATNIYIFSLALAGALVTTTMPFQSTDYLMNSWPFGDVLCKIVISTDYYSMFTSIFTLTMMCVDRYIAVCHPVKALDFRTPLKAKIINICIWLLSSSVGISAIVLGGTKVREDVDVIECSLQFPDDDYSWWDLFMKICVFIFAFVIPVLIIIVCYTLMILRLKSVRLLSGSREKDRNLRRITRLVLVVVAVFVVCWTPIHIFILVEALGSTSHSTAALSSYYFCIALGYINSSLNPILYAFLDENFKRCFRDFCFPLKMRMKRQSTSRVRNTVQDPAYLRDIDGMDKPV